European Patent Application EP 4 227 414 A1, published August 16, 2023. Title: 新型PiggyBac转座子系统及其用途. Applicant: 上海君赛生物科技有限公司. The sequence listing filed with the application follows.

SEQUENCE LISTING (45 sequences)

SEQ ID NO: 1 - DNA, 67 bp, Artificial Sequence
  3IPR
ttaaccctagaaagataatcatattgtgacgtacgttaaagataatcatgcgtaaaattgacgcatg

SEQ ID NO: 2 - DNA, 18 bp, Artificial Sequence
  MCS
tctagagaattcgtcgac

SEQ ID NO: 3 - DNA, 225 bp, Artificial Sequence
  bGH polyA
ctgtgccttctagttgccagccatctgttgtttgcccctcccccgtgccttccttgaccctggaaggtgccactcccactgtcctttcctaataaaatgaggaaattgcatcgcattgtctgagtaggtgtcattctattctggggggtggggtggggcaggacagcaagggggaggattgggaagacaatagcaggcatgctggggatgcggtgggctctatgg

SEQ ID NO: 4 - DNA, 193 bp, Artificial Sequence
  Enhancer
tgtggaaagtccccaggctccccagcaggcagaagtatgcaaagcatgcatctcaattagtcagcaaccaggtgtggaaagtccccaggctccccagcaggcagaagtatgcaaagcatgcatctcaattagtcagcaaccattgagctggggactttccagctggggactttccagctggggactttccagg

SEQ ID NO: 5 - DNA, 103 bp, Artificial Sequence
  insulator
agagaaatgttctggcacctgcacttgcactggggacagcctattttgctagtttgttttgtttcgttttgttttgatggagagcgtatgttagtactatcga

SEQ ID NO: 6 - DNA, 40 bp, Artificial Sequence
  5ITR
gcatgcgtcaattttacgcagactatctttctagggttaa

SEQ ID NO: 7 - DNA, 1842 bp, Artificial Sequence
  PB
atgggcaaacctaagaaaatcaaaacagaagatggcagcagcctggacgacgagcacatcctgagcgccctgctgcagagcgacgacgagctggtgggcgaggacagcgacagcgaggtgagcgaccacgtgagcgaggacgacgtgcagagcgacaccgaggaggccttcatcgacgaggtgcacgaggtgcagcccaccagcagcggcagcgagatcctggacgagcagaacgtgatcgagcagcccggcagcagcctggccagcaaccgcatcctgaccctgccccagcgcaccatccgcggcaagaacaagcactgctggagcaccagcaagcccacccgccgcagccgcgtgagcgccctgaacatcgtgcgcagccagcgcggccccacccgcatgtgccgcaacatctacgaccccctgctgtgcttcaagctgttcttcaccgacgagatcatcagcgagatcgtgaagtggaccaacgccgagatcagcctgaagcgccgcgagagcatgaccagcgccaccttccgcgacaccaacgaggacgagatctacgccttcttcggcatcctggtgatgaccgccgtgcgcaaggacaaccacatgagcaccgacgacctgttcgaccgcagcctgagcatggtgtacgtgagcgtgatgagccgcgaccgcttcgacttcctgatccgctgcctgcgcatggacgacaagagcatccgccccaccctgcgcgagaacgacgtgttcacccccgtgcgcaagatctgggacctgttcatccaccagtgcatccagaactacacccccggcgcccacctgaccatcgacgagcagctgctgggcttccgcggccgctgccccttccgcgtgtacatccccaacaagcccagcaagtacggcatcaagatcctgatgatgtgcgacagcggcaccaagtacatgatcaacggcatgccctacctgggccgcggcacccagaccaacggcgtgcccctgggcgagtactacgtgaaggagctgagcaagcccgtgcacggcagctgccgcaacatcacctgcgacaactggttcaccagcatccccctggccaagaacctgctgcaggagccctacaagctgaccatcgtgggcaccgtgcgcagcaacaagcgcgagatccccgaggtgctgaagaacagccgcagccgccccgtgggcaccagcatgttctgcttcgacggccccctgaccctggtgagctacaagcccaagcccgccaagatggtgtacctgctgagcagctgcgacgaggacgccagcatcaacgagagcaccggcaagccccagatggtgatgtactacaaccagaccaagggcggcgtggacaccctggaccagatgtgcagcgtgatgacctgcagccgcaagaccaaccgctggcccatggccctgctgtacggcatgatcaacatcgcctgcatcaacagcttcatcatctacagccacaacgtgagcagcaagggcgagaaggtgcagagccgcaagaagttcatgcgcaacctgtacatgggcctgaccagcagcttcatgcgcaagcgcctggaggcccccaccctgaagcgctacctgcgcgacaacatcagcaacatcctgcccaaggaggtgcccggcaccagcgacgacagcaccgaggagcccgtgatgaagaagcgcacctactgcacctactgccccagcaagatccgccgcaaggccagcgccagctgcaagaagtgcaagaaggtgatctgccgcgagcacaacatcgacatgtgccagagctgcttccctgctgccaagagggtcaagttggactaa

SEQ ID NO: 8 - DNA, 45 bp, Artificial Sequence
  5UTR
gcttgttctttttgcagaagctcagaataaacgctcaactttggc

SEQ ID NO: 9 - DNA, 39 bp, Artificial Sequence
  promoter
ggtaggcgtgtacggtgggaggcctatataagcagagct

SEQ ID NO: 10 - DNA, 2630 bp, Artificial Sequence
  Nucleic acid construct
ttaaccctagaaagataatcatattgtgacgtacgttaaagataatcatgcgtaaaattgacgcatgtctagagaattcgtcgacctgtgccttctagttgccagccatctgttgtttgcccctcccccgtgccttccttgaccctggaaggtgccactcccactgtcctttcctaataaaatgaggaaattgcatcgcattgtctgagtaggtgtcattctattctggggggtggggtggggcaggacagcaagggggaggattgggaagacaatagcaggcatgctggggatgcggtgggctctatggtgtggaaagtccccaggctccccagcaggcagaagtatgcaaagcatgcatctcaattagtcagcaaccaggtgtggaaagtccccaggctccccagcaggcagaagtatgcaaagcatgcatctcaattagtcagcaaccattgagctggggactttccagctggggactttccagctggggactttccaggagagaaatgttctggcacctgcacttgcactggggacagcctattttgctagtttgttttgtttcgttttgttttgatggagagcgtatgttagtactatcgacacacaaaaaaccaacacacagatctaatgaaaataaagatcttttattgcatgcgtcaattttacgcagactatctttctagggttaaatcgatttagtccaacttgaccctcttggcagcagggaagcagctctggcacatgtcgatgttgtgctcgcggcagatcaccttcttgcacttcttgcagctggcgctggccttgcggcggatcttgctggggcagtaggtgcagtaggtgcgcttcttcatcacgggctcctcggtgctgtcgtcgctggtgccgggcacctccttgggcaggatgttgctgatgttgtcgcgcaggtagcgcttcagggtgggggcctccaggcgcttgcgcatgaagctgctggtcaggcccatgtacaggttgcgcatgaacttcttgcggctctgcaccttctcgcccttgctgctcacgttgtggctgtagatgatgaagctgttgatgcaggcgatgttgatcatgccgtacagcagggccatgggccagcggttggtcttgcggctgcaggtcatcacgctgcacatctggtccagggtgtccacgccgcccttggtctggttgtagtacatcaccatctggggcttgccggtgctctcgttgatgctggcgtcctcgtcgcagctgctcagcaggtacaccatcttggcgggcttgggcttgtagctcaccagggtcagggggccgtcgaagcagaacatgctggtgcccacggggcggctgcggctgttcttcagcacctcggggatctcgcgcttgttgctgcgcacggtgcccacgatggtcagcttgtagggctcctgcagcaggttcttggccagggggatgctggtgaaccagttgtcgcaggtgatgttgcggcagctgccgtgcacgggcttgctcagctccttcacgtagtactcgcccaggggcacgccgttggtctgggtgccgcggcccaggtagggcatgccgttgatcatgtacttggtgccgctgtcgcacatcatcaggatcttgatgccgtacttgctgggcttgttggggatgtacacgcggaaggggcagcggccgcggaagcccagcagctgctcgtcgatggtcaggtgggcgccgggggtgtagttctggatgcactggtggatgaacaggtcccagatcttgcgcacgggggtgaacacgtcgttctcgcgcagggtggggcggatgctcttgtcgtccatgcgcaggcagcggatcaggaagtcgaagcggtcgcggctcatcacgctcacgtacaccatgctcaggctgcggtcgaacaggtcgtcggtgctcatgtggttgtccttgcgcacggcggtcatcaccaggatgccgaagaaggcgtagatctcgtcctcgttggtgtcgcggaaggtggcgctggtcatgctctcgcggcgcttcaggctgatctcggcgttggtccacttcacgatctcgctgatgatctcgtcggtgaagaacagcttgaagcacagcagggggtcgtagatgttgcggcacatgcgggtggggccgcgctggctgcgcacgatgttcagggcgctcacgcggctgcggcgggtgggcttgctggtgctccagcagtgcttgttcttgccgcggatggtgcgctggggcagggtcaggatgcggttgctggccaggctgctgccgggctgctcgatcacgttctgctcgtccaggatctcgctgccgctgctggtgggctgcacctcgtgcacctcgtcgatgaaggcctcctcggtgtcgctctgcacgtcgtcctcgctcacgtggtcgctcacctcgctgtcgctgtcctcgcccaccagctcgtcgtcgctctgcagcagggcgctcaggatgtgctcgtcgtccaggctgctgccatcttctgttttgattttcttaggtttgcccatggtgccaaagttgagcgtttattctgagcttctgcaaaaagaacaagcagctctgcttatataggcctcccaccgtacacgcctacc

SEQ ID NO: 11 - DNA, 586 bp, Artificial Sequence
  promoter
ttgaggaatttccattgaggaatttccattgaggaatttccaggatctgcgatcgctccggtgcccgtcagtgggcagagcgcacatcgcccacagtccccgagaagttggggggaggggtcggcaattgaacgggtgcctagagaaggtggcgcggggtaaactgggaaagtgatgtcgtgtactggctccgcctttttcccgagggtgggggagaaccgtatataagtgcagtagtcgccgtgaacgttctttttcgcaacgggtttgccgccagaacacagctgaagcttcgaggggctcgcatctctccttcacgcgcccgccgccctacctgaggccgccatccacgccggttgagtcgcgttctgccgcctcccgcctgtggtgcctcctgaactgcgtccgccgtctaggtaagtttaaagctcaggtcgagaccgggcctttgtccggcgctcccttggagcctacctagactcagccggctctccacgctttgcctgaccctgcttgctcaactctacgtctttgtttcgttttctgttctgcgccgttacagatccaagctgtgaccggcgcctac

SEQ ID NO: 12 - DNA, 726 bp, Artificial Sequence
  EGFP
gccaccatggtgagcaagggcgaggagctgttcaccggggtggtgcccatcctggtcgagctggacggcgacgtaaacggccacaagttcagcgtgtccggcgagggcgagggcgatgccacctacggcaagctgaccctgaagttcatctgcaccaccggcaagctgcccgtgccctggcccaccctcgtgaccaccctgacctacggcgtgcagtgcttcagccgctaccccgaccacatgaagcagcacgacttcttcaagtccgccatgcccgaaggctacgtccaggagcgcaccatcttcttcaaggacgacggcaactacaagacccgcgccgaggtgaagttcgagggcgacaccctggtgaaccgcatcgagctgaagggcatcgacttcaaggaggacggcaacatcctggggcacaagctggagtacaactacaacagccacaacgtctatatcatggccgacaagcagaagaacggcatcaaggtgaacttcaagatccgccacaacatcgaggacggcagcgtgcagctcgccgaccactaccagcagaacacccccatcggcgacggccccgtgctgctgcccgacaaccactacctgagcacccagtccgccctgagcaaagaccccaacgagaagcgcgatcacatggtcctgctggagttcgtgaccgccgccgggatcactctcggcatggacgagctgtacaagtga

SEQ ID NO: 13 - DNA, 222 bp, Artificial Sequence
  SV40 polyA
cagacatgataagatacattgatgagtttggacaaaccacaactagaatgcagtgaaaaaaatgctttatttgtgaaatttgtgatgctattgctttatttgtaaccattataagctgcaataaacaagttaacaacaacaattgcattcattttatgtttcaggttcagggggaggtgtgggaggttttttaaagcaagtaaaacctctacaaatgtggta

SEQ ID NO: 14 - DNA, 2850 bp, Artificial Sequence
  Nucleic acid construct
ttaaccctagaaagataatcatattgtgacgtacgttaaagataatcatgcgtaaaattgacgcatgtctagagaattcgtcgacctgtgccttctagttgccagccatctgttgtttgcccctcccccgtgccttccttgaccctggaaggtgccactcccactgtcctttcctaataaaatgaggaaattgcatcgcattgtctgagtaggtgtcattctattctggggggtggggtggggcaggacagcaagggggaggattgggaagacaatagcaggcatgctggggatgcggtgggctctatggtgtggaaagtccccaggctccccagcaggcagaagtatgcaaagcatgcatctcaattagtcagcaaccaggtgtggaaagtccccaggctccccagcaggcagaagtatgcaaagcatgcatctcaattagtcagcaaccattgagctggggactttccagctggggactttccagctggggactttccaggagagaaatgttctggcacctgcacttgcactggggacagcctattttgctagtttgttttgtttcgttttgttttgatggagagcgtatgttagtactatcgacacacaaaaaaccaacacacagatctaatgaaaataaagatcttttattgcatgcgtcaattttacgcagactatctttctagggttaaatcgatggtaggcgtgtacggtgggaggcctatataagcagagctgcttgttctttttgcagaagctcagaataaacgctcaactttggcaccatgggcaaacctaagaaaatcaaaacagaagatggcagcagcctggacgacgagcacatcctgagcgccctgctgcagagcgacgacgagctggtgggcgaggacagcgacagcgaggtgagcgaccacgtgagcgaggacgacgtgcagagcgacaccgaggaggccttcatcgacgaggtgcacgaggtgcagcccaccagcagcggcagcgagatcctggacgagcagaacgtgatcgagcagcccggcagcagcctggccagcaaccgcatcctgaccctgccccagcgcaccatccgcggcaagaacaagcactgctggagcaccagcaagcccacccgccgcagccgcgtgagcgccctgaacatcgtgcgcagccagcgcggccccacccgcatgtgccgcaacatctacgaccccctgctgtgcttcaagctgttcttcaccgacgagatcatcagcgagatcgtgaagtggaccaacgccgagatcagcctgaagcgccgcgagagcatgaccagcgccaccttccgcgacaccaacgaggacgagatctacgccttcttcggcatcctggtgatgaccgccgtgcgcaaggacaaccacatgagcaccgacgacctgttcgaccgcagcctgagcatggtgtacgtgagcgtgatgagccgcgaccgcttcgacttcctgatccgctgcctgcgcatggacgacaagagcatccgccccaccctgcgcgagaacgacgtgttcacccccgtgcgcaagatctgggacctgttcatccaccagtgcatccagaactacacccccggcgcccacctgaccatcgacgagcagctgctgggcttccgcggccgctgccccttccgcgtgtacatccccaacaagcccagcaagtacggcatcaagatcctgatgatgtgcgacagcggcaccaagtacatgatcaacggcatgccctacctgggccgcggcacccagaccaacggcgtgcccctgggcgagtactacgtgaaggagctgagcaagcccgtgcacggcagctgccgcaacatcacctgcgacaactggttcaccagcatccccctggccaagaacctgctgcaggagccctacaagctgaccatcgtgggcaccgtgcgcagcaacaagcgcgagatccccgaggtgctgaagaacagccgcagccgccccgtgggcaccagcatgttctgcttcgacggccccctgaccctggtgagctacaagcccaagcccgccaagatggtgtacctgctgagcagctgcgacgaggacgccagcatcaacgagagcaccggcaagccccagatggtgatgtactacaaccagaccaagggcggcgtggacaccctggaccagatgtgcagcgtgatgacctgcagccgcaagaccaaccgctggcccatggccctgctgtacggcatgatcaacatcgcctgcatcaacagcttcatcatctacagccacaacgtgagcagcaagggcgagaaggtgcagagccgcaagaagttcatgcgcaacctgtacatgggcctgaccagcagcttcatgcgcaagcgcctggaggcccccaccctgaagcgctacctgcgcgacaacatcagcaacatcctgcccaaggaggtgcccggcaccagcgacgacagcaccgaggagcccgtgatgaagaagcgcacctactgcacctactgccccagcaagatccgccgcaaggccagcgccagctgcaagaagtgcaagaaggtgatctgccgcgagcacaacatcgacatgtgccagagctgcttccctgctgccaagagggtcaagttggactaacagacatgataagatacattgatgagtttggacaaaccacaactagaatgcagtgaaaaaaatgctttatttgtgaaatttgtgatgctattgctttatttgtaaccattataagctgcaataaacaagttaacaacaacaattgcattcattttatgtttcaggttcagggggaggtgtgggaggttttttaaagcaagtaaaacctctacaaatgtgg

SEQ ID NO: 15 - DNA, 48 bp, Artificial Sequence
  insulator
aacatacgctctccatcaaaacaaaacgaaacaaaacaaactagcaaa

SEQ ID NO: 16 - DNA, 49 bp, Artificial Sequence
  polyA
aataaaagatctttattttcattagatctgtgtgttggttttttgtgtg

SEQ ID NO: 17 - DNA, 62 bp, Artificial Sequence
  5UTR
cactcctccccatcctctccctctgtccctctgtccctctgaccctgcactgtcccagcacc

SEQ ID NO: 18 - DNA, 111 bp, Artificial Sequence
  5UTR
acagagtaaacttttgctgggctccaagtgaccgcccatagtttattataaaggtgactgcaccctgcagccaccagcactgcctggctccacgtgcctcctggtctcagt

SEQ ID NO: 19 - DNA, 111 bp, Artificial Sequence; identical to SEQ ID NO: 18
  5UTR

SEQ ID NO: 20 - DNA, 58 bp, Artificial Sequence
  5UTR
agcaatcctttctttcagctggagtgctcctcaggagccagccccacccttagaaaag

SEQ ID NO: 21 - DNA, 121 bp, Artificial Sequence
  5UTR
cggaagcccatccaccaatcctcacctctcacctctgtgtccgccctgctgggaaatattccaggctttggccaaggccagtgcagccccaggttcccgagcggcaggttgggtgcggacc

SEQ ID NO: 22 - DNA, 111 bp, Artificial Sequence
  5UTR
gacgccatcccggccagaaaagccctggccagtggcgggcgcgacactatccgtgcggccaggcggagacccggaggaccgaagcttccggacgacgaggaaccgcccaac

SEQ ID NO: 23 - DNA, 58 bp, Artificial Sequence
  5UTR
aggcacagacaccaaggacagagacgctggctaggccgccctccccactgttaccaac

SEQ ID NO: 24 - DNA, 73 bp, Artificial Sequence
  5UTR
agtatattagtgctaatttccctccgtttgtcctagcttttctcttctgtcaaccccacacgcctttggcaca

SEQ ID NO: 25 - DNA, 360 bp, Artificial Sequence
  Enhancer
gcgttacataacttacggtaaatggcccgcctggctgaccgcccaacgacccattgaccaataatgacgtatgttcccatagtaacgccaatagggactttccattgacgtcaatgggtggagtatttacggtaaactgcccacttggcagtacatcaagtgtatcatatgccaagtacgccccctattgacgtcaatgacggtaaatggccgcctggcattatgcccagtacatgaccttatgggactttctacttggcagtacatctacgtattagtcatcgctattaccatggtgatgcggttttggcagtacatcaatgggcgtggatagcggtttgactcacggggatttccaag

SEQ ID NO: 26 - DNA, 116 bp, Artificial Sequence
  Enhancer
cttctgaggcggaaagaaccagctgtggaatgtgtgtcagttagggtgtggaaagtccccaggctccccagcaggcagaagtatgcaaagcatgcatctcaattagtcagcaacca

SEQ ID NO: 27 - DNA, 60 bp, Artificial Sequence
  Enhancer
ctcaagcacagcaatgctgagtcatgatgagtcatgctgaggcttagggtgtgtgcccag

SEQ ID NO: 28 - DNA, 242 bp, Artificial Sequence
  Enhancer
agggacagcccccccccaaagcccccagggatgtaattacgtccctcccccgctagggcagcagcgagccgcccggggctccggtccggtccggcgctcccccgcatccccgagccggcagcgtgcggggacagcccgggcacggggaaggtggcacgggatcgctttcctctgaacgcttctcgctgctctttgagcctgcagacacctggggggatacggggaaaaaagctttaggctga

SEQ ID NO: 29 - DNA, 20 bp, Artificial Sequence
  primer
ggacgagatctacgccttct

SEQ ID NO: 30 - DNA, 20 bp, Artificial Sequence
  primer
ctcatcacgctcacgtacac

SEQ ID NO: 31 - DNA, 20 bp, Artificial Sequence
  probe
tgcgcacggcggtcatcacc

SEQ ID NO: 32 - DNA, 20 bp, Artificial Sequence
  primer
gggacctgactgactacctc

SEQ ID NO: 33 - DNA, 20 bp, Artificial Sequence
  primer
aatgtcacgcacgatttccc

SEQ ID NO: 34 - DNA, 20 bp, Artificial Sequence
  probe
caccgagcgcggctacagct

SEQ ID NO: 35 - DNA, 27 bp, Artificial Sequence
  NLS
cctgctgccaagagggtcaagttggac

SEQ ID NO: 36 - protein, 613 aa, Artificial Sequence
  PB
MGKPKKIKTEDGSSLDDEHILSALLQSDDELVGEDSDSEVSDHVSEDDVQSDTEEAFIDEVHEVQPTSSGSEILDEQNVIEQPGSSLASNRILTLPQRTIRGKNKHCWSTSKPTRRSRVSALNIVRSQRGPTRMCRNIYDPLLCFKLFFTDEIISEIVKWTNAEISLKRRESMTSATFRDTNEDEIYAFFGILVMTAVRKDNHMSTDDLFDRSLSMVYVSVMSRDRFDFLIRCLRMDDKSIRPTLRENDVFTPVRKIWDLFIHQCIQNYTPGAHLTIDEQLLGFRGRCPFRVYIPNKPSKYGIKILMMCDSGTKYMINGMPYLGRGTQTNGVPLGEYYVKELSKPVHGSCRNITCDNWFTSIPLAKNLLQEPYKLTIVGTVRSNKREIPEVLKNSRSRPVGTSMFCFDGPLTLVSYKPKPAKMVYLLSSCDEDASINESTGKPQMVMYYNQTKGGVDTLDQMCSVMTCSRKTNRWPMALLYGMINIACINSFIIYSHNVSSKGEKVQSRKKFMRNLYMGLTSSFMRKRLEAPTLKRYLRDNISNILPKEVPGTSDDSTEEPVMKKRTYCTYCPSKIRRKASASCKKCKKVICREHNIDMCQSCFPAAKRVKLD

SEQ ID NO: 37 - DNA, 76 bp, Artificial Sequence
  promoter
caacaaaatgtcgtaacaagggcggtaggcgtgtacggtgggaggtctatataagcagagctcgtttagtgaaccg

SEQ ID NO: 38 - DNA, 203 bp, Artificial Sequence
  promoter
tgcatctcaattagtcagcaaccatagtcccgcccctaactccgcccatcccgcccctaactccgcccagttccgcccattctccgccccatcgctgactaattttttttatttatgcagaggccgaggccgcctcggcctctgagctattccagaagtagtgaggaggcttttttggaggcctaggcttttgcaaaaagctt

SEQ ID NO: 39 - DNA, 63 bp, Artificial Sequence
  promoter
ttcgcatattaaggtgacgcgtgtggcctcgaacaccgagcgaccctgcagcgacccgcttaa

SEQ ID NO: 40 - DNA, 41 bp, Artificial Sequence
  promoter
ggggggctataaaagggggtgggggcgttcgtcctcactct

SEQ ID NO: 41 - DNA, 178 bp, Artificial Sequence
  promoter
ctgacaaattcagtataaaagcttggggctggggccgagcactggggactttgagggtggccaggccagcgtaggaggccagcgtaggatcctgctgggagcggggaactgagggaagcgacgccgagaaagcaggcgtaccacggagggagagaaaagctccggaagcccagcagcg

SEQ ID NO: 42 - DNA, 25 bp, Artificial Sequence
  promoter
tctagagggtatataatgggggcca

SEQ ID NO: 43 - DNA, 1461 bp, Artificial Sequence
  HER2CAR
gccaccatggccttaccagtgaccgccttgctcctgccgctggccttgctgctccacgccgccaggccggacatccagatgacccagtccccttcctccctctctgcctctgtgggagaccgcgttaccatcacatgccgagcttcccaggacgtgaacacagccgtggcctggtaccagcagaagcccgggaaggcacccaaactcctcatctactccgcctccttcctagagagtggcgtgccttcccgattctccggctccaggagtggcacggactttacgctcaccattagtagcctgcagcccgaagacttcgcgacctactattgtcagcaacactacacgacgccaccaactttcggccagggtaccaaggtcgagattaagcgaaccggcagtaccagtgggtctggcaagcccggcagcggcgagggatccgaggtccagctggtcgagtccggcgggggcctggtgcagccgggcggctcgctgaggttatcttgcgccgccagtggcttcaacatcaaggatacttacatccactgggtgaggcaggctccgggcaagggcctggaatgggtggctaggatctaccctactaacgggtacacacgctacgcagattcggtgaaaggccgcttcactatctccgccgacacctcgaagaacactgcttacctgcagatgaactccctcagggccgaagatactgcagtctactactgctcccgctggggtggggacggcttcgtagccatggacgtgtggggtcagggcactctagttacagtgtcatccattgaagttatgtatcctcctccttacctagacaatgagaagagcaatggaaccattatccatgtgaaagggaaacacctttgtccaagtcccctatttcccggaccttctaagcccttttgggtgctggtggtggttggtggagtcctggcttgctatagcttgctagtaacagtgaggcctttattattttctgggtgaggagtaagaggagcaggctcctgcacagtgactacatgaacatgactccccgccgccccgggcccacccgcaagcattaccagccctatgccccaccacgcgacttcgcagcctatcgctccagagtgaagttcagcaggagcgcagacgcccccgcgtaccagcagggccagaaccagctctataacgagctcaatctaggacgaagagaggagtacgatgttttggacaagagacgtggccgggaccctgagatggggggaaagccgagaaggaagaaccctcaggaaggcctgtacaatgaactgcaaagataagatggcggaggcctacagtgagattgggatgaaaggcgagcgccggaggggcaaggggcacgatggcctttaccagggtctcagtacagccaccaaggacacctacgacgcccttcacatgcaggccctgccccctcgctga

SEQ ID NO: 44 - DNA, 1836 bp, Artificial Sequence
  NY-ESO-1-TCR
atggagaccctcttgggcctgcttatcctttggctgcagctgcaatgggtgagcagcaaacaggaggtgacgcagattcctgcagctctgagtgtcccagaaggagaaaacttggttctcaactgcagtttcactgatagcgctatttacaacctccagtggtttaggcaggaccctgggaaaggtctcacatctctgttgcttattcagtcaagtcagagagagcaaacaagtggaagacttaatgcctcgctggataaatcatcaggacgtagtactttatacattgcagcttctcagcctggtgactcagccacctacctctgtgctgtgaggcccacatcaggaggaagctacatacctacatttggaagaggaaccagccttattgttcatccggatatccagaaccctgaccctgccgtgtaccagctgagagactctaaatccagtgacaagtctgtctgcctattcaccgattttgattctcaaacaaatgtgtcacaaagtaaggattctgatgtgtatatcacagacaaaactgtgctagacatgaggtctatggacttcaagagcaacagtgctgtggcctggagcaacaaatctgactttgcatgtgcaaacgccttcaacaacagcattattccagaagacaccttcttccccagcccagaaagttcctgtgatgtcaagctggtcgagaaaagctttgaaacagatacgaacctaaactttcaaaacctgtcagtgattgggttccgaatcctcctcctgaaagtggccgggtttaatctgctcatgacgctgcggctgtggtccagcgccaccaacttcagcctgctgaagcaggccggcgacgtggaggagaaccccggccccatgagcatcggcctcctgtgctgtgcagccttgtctctcctgtgggcaggtccagtgaatgctggtgtcactcagaccccaaaattccaggtcctgaagacaggacagagcatgacactgcagtgtgcccaggatatgaaccatgaatacatgtcctggtatcgacaagacccaggcatggggctgaggctgattcattactcagttggtgctggtatcactgaccaaggagaagtccccaatggctacaatgtctccagatcaaccacagaggatttcccgctcaggctgctgtcggctgctccctcccagacatctgtgtacttctgtgccagcagttacgtcgggaacaccggggagctgttttttggagaaggctctaggctgaccgtactggaggacctgaaaaacgtgttcccacccgaggtcgctgtgtttgagccatcagaagcagagatctcccacacccaaaaggccacactggtatgcctggccacaggcttctaccccgaccacgtggagctgagctggtgggtgaatgggaaggaggtgcacagtggggtcagcacagacccgcagcccctcaaggagcagcccgccctcaatgactccagatactgcctgagcagccgcctgagggtctcggccaccttctggcagaacccccgcaaccacttccgctgtcaagtccagttctacgggctctcggagaatgacgagtggacccaggatagggccaaacccgtcacccagatcgtcagcgccgaggcctggggtagagcagactgtggcttcacctccgagtcttaccagcaaggggtcctgtctgccaccatcctctatgagatcttgctagggaaggccaccttgtatgccgtgctggtcagtgccctcgtgctgatggctatggtcaagagaaaggattccagaggccgggccaagcggtccggatccgga

SEQ ID NO: 45 - DNA, 2610 bp, Artificial Sequence
  NY-ESO-1-TCR-EGFP
atggagaccctcttgggcctgcttatcctttggctgcagctgcaatgggtgagcagcaaacaggaggtgacgcagattcctgcagctctgagtgtcccagaaggagaaaacttggttctcaactgcagtttcactgatagcgctatttacaacctccagtggtttaggcaggaccctgggaaaggtctcacatctctgttgcttattcagtcaagtcagagagagcaaacaagtggaagacttaatgcctcgctggataaatcatcaggacgtagtactttatacattgcagcttctcagcctggtgactcagccacctacctctgtgctgtgaggcccacatcaggaggaagctacatacctacatttggaagaggaaccagccttattgttcatccggatatccagaaccctgaccctgccgtgtaccagctgagagactctaaatccagtgacaagtctgtctgcctattcaccgattttgattctcaaacaaatgtgtcacaaagtaaggattctgatgtgtatatcacagacaaaactgtgctagacatgaggtctatggacttcaagagcaacagtgctgtggcctggagcaacaaatctgactttgcatgtgcaaacgccttcaacaacagcattattccagaagacaccttcttccccagcccagaaagttcctgtgatgtcaagctggtcgagaaaagctttgaaacagatacgaacctaaactttcaaaacctgtcagtgattgggttccgaatcctcctcctgaaagtggccgggtttaatctgctcatgacgctgcggctgtggtccagcgccaccaacttcagcctgctgaagcaggccggcgacgtggaggagaaccccggccccatgagcatcggcctcctgtgctgtgcagccttgtctctcctgtgggcaggtccagtgaatgctggtgtcactcagaccccaaaattccaggtcctgaagacaggacagagcatgacactgcagtgtgcccaggatatgaaccatgaatacatgtcctggtatcgacaagacccaggcatggggctgaggctgattcattactcagttggtgctggtatcactgaccaaggagaagtccccaatggctacaatgtctccagatcaaccacagaggatttcccgctcaggctgctgtcggctgctccctcccagacatctgtgtacttctgtgccagcagttacgtcgggaacaccggggagctgttttttggagaaggctctaggctgaccgtactggaggacctgaaaaacgtgttcccacccgaggtcgctgtgtttgagccatcagaagcagagatctcccacacccaaaaggccacactggtatgcctggccacaggcttctaccccgaccacgtggagctgagctggtgggtgaatgggaaggaggtgcacagtggggtcagcacagacccgcagcccctcaaggagcagcccgccctcaatgactccagatactgcctgagcagccgcctgagggtctcggccaccttctggcagaacccccgcaaccacttccgctgtcaagtccagttctacgggctctcggagaatgacgagtggacccaggatagggccaaacccgtcacccagatcgtcagcgccgaggcctggggtagagcagactgtggcttcacctccgagtcttaccagcaaggggtcctgtctgccaccatcctctatgagatcttgctagggaaggccaccttgtatgccgtgctggtcagtgccctcgtgctgatggctatggtcaagagaaaggattccagaggccgggccaagcggtccggatccggagccaccaacttcagcctgctgaagcaggccggcgacgtggaggagaaccccggccccatgtccaagggcgaggaactgttcacgggcgtcgtcccgatcctcgtcgaactcgatggcgacgtcaacggccacaagttctccgtcagcggtgaaggtgaaggcgacgccacctacggcaagctcacccttaagttcatctgcaccaccggcaaactgccggtgccgtggccgacgctggtcacgaccctcacgtatggcgttcagtgcttctcgcgctacccggaccacatgaagcagcacgatttcttcaagtcggcgatgccggaaggctacgtccaggaacgcacgatcttcttcaaggacgatggcaactacaagacccgcgccgaagtcaagttcgagggcgacacgcttgtgaatcgcatcgaacttaagggcatcgacttcaaggaagatggcaacatcctcggccacaagctggagtataactacaattcgcacaacgtctacatcatggctgacaagcagaagaatggtatcaaggttaacttcaagatccgccacaacatcgaagacggctccgtccagctggcggaccactatcagcagaacaccccgatcggcgacggcccggttctcctcccggataaccactacctcagcacgcagtcggcgctgtcgaaggacccgaatgaaaagcgcgaccacatggtccttctggagttcgtgaccgcggcgggcatcacgcacggcatggacgaactttacaagtaa